European Patent Application EP 4 786 484 A1, published August 5, 2026. Title: 环肽化合物及其应用. Applicant: 深圳众格生物科技有限公司. The sequence listing filed with the application follows.

SEQUENCE LISTING (729 sequences)

SEQ ID NO: 1 - protein, 6 aa, synthetic construct
  source 1..6: note = ring structure
AAAGHK

SEQ ID NO: 2 - protein, 6 aa, synthetic construct
  source 1..6: note = ring structure
AAGGHK

SEQ ID NO: 3 - protein, 6 aa, synthetic construct
  source 1..6: note = ring structure
AAIGHK

SEQ ID NO: 4 - protein, 6 aa, synthetic construct
  source 1..6: note = ring structure
AALGHK

SEQ ID NO: 5 - protein, 6 aa, synthetic construct
  source 1..6: note = ring structure
AAMGHK

SEQ ID NO: 6 - protein, 6 aa, synthetic construct
  source 1..6: note = ring structure
AAFGHK

SEQ ID NO: 7 - protein, 6 aa, synthetic construct
  source 1..6: note = ring structure
AAPGHK

SEQ ID NO: 8 - protein, 6 aa, synthetic construct
  source 1..6: note = ring structure
AAWGHK

SEQ ID NO: 9 - protein, 6 aa, synthetic construct
  source 1..6: note = ring structure
AAVGHK

SEQ ID NO: 10 - protein, 6 aa, synthetic construct
  source 1..6: note = ring structure
AGAGHK

SEQ ID NO: 11 - protein, 6 aa, synthetic construct
  source 1..6: note = ring structure
AGGGHK

SEQ ID NO: 12 - protein, 6 aa, synthetic construct
  source 1..6: note = ring structure
AGIGHK

SEQ ID NO: 13 - protein, 6 aa, synthetic construct
  source 1..6: note = ring structure
AGLGHK

SEQ ID NO: 14 - protein, 6 aa, synthetic construct
  source 1..6: note = ring structure
AGMGHK

SEQ ID NO: 15 - protein, 6 aa, synthetic construct
  source 1..6: note = ring structure
AGFGHK

SEQ ID NO: 16 - protein, 6 aa, synthetic construct
  source 1..6: note = ring structure
AGPGHK

SEQ ID NO: 17 - protein, 6 aa, synthetic construct
  source 1..6: note = ring structure
AGWGHK

SEQ ID NO: 18 - protein, 6 aa, synthetic construct
  source 1..6: note = ring structure
AGVGHK

SEQ ID NO: 19 - protein, 6 aa, synthetic construct
  source 1..6: note = ring structure
AIAGHK

SEQ ID NO: 20 - protein, 6 aa, synthetic construct
  source 1..6: note = ring structure
AIGGHK

SEQ ID NO: 21 - protein, 6 aa, synthetic construct
  source 1..6: note = ring structure
AIIGHK

SEQ ID NO: 22 - protein, 6 aa, synthetic construct
  source 1..6: note = ring structure
AILGHK

SEQ ID NO: 23 - protein, 6 aa, synthetic construct
  source 1..6: note = ring structure
AIMGHK

SEQ ID NO: 24 - protein, 6 aa, synthetic construct
  source 1..6: note = ring structure
AIFGHK

SEQ ID NO: 25 - protein, 6 aa, synthetic construct
  source 1..6: note = ring structure
AIPGHK

SEQ ID NO: 26 - protein, 6 aa, synthetic construct
  source 1..6: note = ring structure
AIWGHK

SEQ ID NO: 27 - protein, 6 aa, synthetic construct
  source 1..6: note = ring structure
AIVGHK

SEQ ID NO: 28 - protein, 6 aa, synthetic construct
  source 1..6: note = ring structure
ALAGHK

SEQ ID NO: 29 - protein, 6 aa, synthetic construct
  source 1..6: note = ring structure
ALGGHK

SEQ ID NO: 30 - protein, 6 aa, synthetic construct
  source 1..6: note = ring structure
ALIGHK

SEQ ID NO: 31 - protein, 6 aa, synthetic construct
  source 1..6: note = ring structure
ALLGHK

SEQ ID NO: 32 - protein, 6 aa, synthetic construct
  source 1..6: note = ring structure
ALMGHK

SEQ ID NO: 33 - protein, 6 aa, synthetic construct
  source 1..6: note = ring structure
ALFGHK

SEQ ID NO: 34 - protein, 6 aa, synthetic construct
  source 1..6: note = ring structure
ALPGHK

SEQ ID NO: 35 - protein, 6 aa, synthetic construct
  source 1..6: note = ring structure
ALWGHK

SEQ ID NO: 36 - protein, 6 aa, synthetic construct
  source 1..6: note = ring structure
ALVGHK

SEQ ID NO: 37 - protein, 6 aa, synthetic construct
  source 1..6: note = ring structure
AMAGHK

SEQ ID NO: 38 - protein, 6 aa, synthetic construct
  source 1..6: note = ring structure
AMGGHK

SEQ ID NO: 39 - protein, 6 aa, synthetic construct
  source 1..6: note = ring structure
AMIGHK

SEQ ID NO: 40 - protein, 6 aa, synthetic construct
  source 1..6: note = ring structure
AMLGHK

SEQ ID NO: 41 - protein, 6 aa, synthetic construct
  source 1..6: note = ring structure
AMMGHK

SEQ ID NO: 42 - protein, 6 aa, synthetic construct
  source 1..6: note = ring structure
AMFGHK

SEQ ID NO: 43 - protein, 6 aa, synthetic construct
  source 1..6: note = ring structure
AMPGHK

SEQ ID NO: 44 - protein, 6 aa, synthetic construct
  source 1..6: note = ring structure
AMWGHK

SEQ ID NO: 45 - protein, 6 aa, synthetic construct
  source 1..6: note = ring structure
AMVGHK

SEQ ID NO: 46 - protein, 6 aa, synthetic construct
  source 1..6: note = ring structure
AFAGHK

SEQ ID NO: 47 - protein, 6 aa, synthetic construct
  source 1..6: note = ring structure
AFGGHK

SEQ ID NO: 48 - protein, 6 aa, synthetic construct
  source 1..6: note = ring structure
AFIGHK

SEQ ID NO: 49 - protein, 6 aa, synthetic construct
  source 1..6: note = ring structure
AFLGHK

SEQ ID NO: 50 - protein, 6 aa, synthetic construct
  source 1..6: note = ring structure
AFMGHK

SEQ ID NO: 51 - protein, 6 aa, synthetic construct
  source 1..6: note = ring structure
AFFGHK

SEQ ID NO: 52 - protein, 6 aa, synthetic construct
  source 1..6: note = ring structure
AFPGHK

SEQ ID NO: 53 - protein, 6 aa, synthetic construct
  source 1..6: note = ring structure
AFWGHK

SEQ ID NO: 54 - protein, 6 aa, synthetic construct
  source 1..6: note = ring structure
AFVGHK

SEQ ID NO: 55 - protein, 6 aa, synthetic construct
  source 1..6: note = ring structure
APAGHK

SEQ ID NO: 56 - protein, 6 aa, synthetic construct
  source 1..6: note = ring structure
APGGHK

SEQ ID NO: 57 - protein, 6 aa, synthetic construct
  source 1..6: note = ring structure
APIGHK

SEQ ID NO: 58 - protein, 6 aa, synthetic construct
  source 1..6: note = ring structure
APLGHK

SEQ ID NO: 59 - protein, 6 aa, synthetic construct
  source 1..6: note = ring structure
APMGHK

SEQ ID NO: 60 - protein, 6 aa, synthetic construct
  source 1..6: note = ring structure
APFGHK

SEQ ID NO: 61 - protein, 6 aa, synthetic construct
  source 1..6: note = ring structure
APPGHK

SEQ ID NO: 62 - protein, 6 aa, synthetic construct
  source 1..6: note = ring structure
APWGHK

SEQ ID NO: 63 - protein, 6 aa, synthetic construct
  source 1..6: note = ring structure
APVGHK

SEQ ID NO: 64 - protein, 6 aa, synthetic construct
  source 1..6: note = ring structure
AWAGHK

SEQ ID NO: 65 - protein, 6 aa, synthetic construct
  source 1..6: note = ring structure
AWGGHK

SEQ ID NO: 66 - protein, 6 aa, synthetic construct
  source 1..6: note = ring structure
AWIGHK

SEQ ID NO: 67 - protein, 6 aa, synthetic construct
  source 1..6: note = ring structure
AWLGHK

SEQ ID NO: 68 - protein, 6 aa, synthetic construct
  source 1..6: note = ring structure
AWMGHK

SEQ ID NO: 69 - protein, 6 aa, synthetic construct
  source 1..6: note = ring structure
AWFGHK

SEQ ID NO: 70 - protein, 6 aa, synthetic construct
  source 1..6: note = ring structure
AWPGHK

SEQ ID NO: 71 - protein, 6 aa, synthetic construct
  source 1..6: note = ring structure
AWWGHK

SEQ ID NO: 72 - protein, 6 aa, synthetic construct
  source 1..6: note = ring structure
AWVGHK

SEQ ID NO: 73 - protein, 6 aa, synthetic construct
  source 1..6: note = ring structure
AVAGHK

SEQ ID NO: 74 - protein, 6 aa, synthetic construct
  source 1..6: note = ring structure
AVGGHK

SEQ ID NO: 75 - protein, 6 aa, synthetic construct
  source 1..6: note = ring structure
AVIGHK

SEQ ID NO: 76 - protein, 6 aa, synthetic construct
  source 1..6: note = ring structure
AVLGHK

SEQ ID NO: 77 - protein, 6 aa, synthetic construct
  source 1..6: note = ring structure
AVMGHK

SEQ ID NO: 78 - protein, 6 aa, synthetic construct
  source 1..6: note = ring structure
AVFGHK

SEQ ID NO: 79 - protein, 6 aa, synthetic construct
  source 1..6: note = ring structure
AVPGHK

SEQ ID NO: 80 - protein, 6 aa, synthetic construct
  source 1..6: note = ring structure
AVWGHK

SEQ ID NO: 81 - protein, 6 aa, synthetic construct
  source 1..6: note = ring structure
AVVGHK

SEQ ID NO: 82 - protein, 6 aa, synthetic construct
  source 1..6: note = ring structure
GAAGHK

SEQ ID NO: 83 - protein, 6 aa, synthetic construct
  source 1..6: note = ring structure
GAGGHK

SEQ ID NO: 84 - protein, 6 aa, synthetic construct
  source 1..6: note = ring structure
GAIGHK

SEQ ID NO: 85 - protein, 6 aa, synthetic construct
  source 1..6: note = ring structure
GALGHK

SEQ ID NO: 86 - protein, 6 aa, synthetic construct
  source 1..6: note = ring structure
GAMGHK

SEQ ID NO: 87 - protein, 6 aa, synthetic construct
  source 1..6: note = ring structure
GAFGHK

SEQ ID NO: 88 - protein, 6 aa, synthetic construct
  source 1..6: note = ring structure
GAPGHK

SEQ ID NO: 89 - protein, 6 aa, synthetic construct
  source 1..6: note = ring structure
GAWGHK

SEQ ID NO: 90 - protein, 6 aa, synthetic construct
  source 1..6: note = ring structure
GAVGHK

SEQ ID NO: 91 - protein, 6 aa, synthetic construct
  source 1..6: note = ring structure
GGAGHK

SEQ ID NO: 92 - protein, 6 aa, synthetic construct
  source 1..6: note = ring structure
GGGGHK

SEQ ID NO: 93 - protein, 6 aa, synthetic construct
  source 1..6: note = ring structure
GGIGHK

SEQ ID NO: 94 - protein, 6 aa, synthetic construct
  source 1..6: note = ring structure
GGLGHK

SEQ ID NO: 95 - protein, 6 aa, synthetic construct
  source 1..6: note = ring structure
GGMGHK

SEQ ID NO: 96 - protein, 6 aa, synthetic construct
  source 1..6: note = ring structure
GGFGHK

SEQ ID NO: 97 - protein, 6 aa, synthetic construct
  source 1..6: note = ring structure
GGPGHK

SEQ ID NO: 98 - protein, 6 aa, synthetic construct
  source 1..6: note = ring structure
GGWGHK

SEQ ID NO: 99 - protein, 6 aa, synthetic construct
  source 1..6: note = ring structure
GGVGHK

SEQ ID NO: 100 - protein, 6 aa, synthetic construct
  source 1..6: note = ring structure
GIAGHK

SEQ ID NO: 101 - protein, 6 aa, synthetic construct
  source 1..6: note = ring structure
GIGGHK

SEQ ID NO: 102 - protein, 6 aa, synthetic construct
  source 1..6: note = ring structure
GIIGHK

SEQ ID NO: 103 - protein, 6 aa, synthetic construct
  source 1..6: note = ring structure
GILGHK

SEQ ID NO: 104 - protein, 6 aa, synthetic construct
  source 1..6: note = ring structure
GIMGHK

SEQ ID NO: 105 - protein, 6 aa, synthetic construct
  source 1..6: note = ring structure
GIFGHK

SEQ ID NO: 106 - protein, 6 aa, synthetic construct
  source 1..6: note = ring structure
GIPGHK

SEQ ID NO: 107 - protein, 6 aa, synthetic construct
  source 1..6: note = ring structure
GIWGHK

SEQ ID NO: 108 - protein, 6 aa, synthetic construct
  source 1..6: note = ring structure
GIVGHK

SEQ ID NO: 109 - protein, 6 aa, synthetic construct
GLAGHK

SEQ ID NO: 110 - protein, 6 aa, synthetic construct
  source 1..6: note = ring structure
GLGGHK

SEQ ID NO: 111 - protein, 6 aa, synthetic construct
  source 1..6: note = ring structure
GLIGHK

SEQ ID NO: 112 - protein, 6 aa, synthetic construct
  source 1..6: note = ring structure
GLLGHK

SEQ ID NO: 113 - protein, 6 aa, synthetic construct
  source 1..6: note = ring structure
GLMGHK

SEQ ID NO: 114 - protein, 6 aa, synthetic construct
  source 1..6: note = ring structure
GLFGHK

SEQ ID NO: 115 - protein, 6 aa, synthetic construct
  source 1..6: note = ring structure
GLPGHK

SEQ ID NO: 116 - protein, 6 aa, synthetic construct
  source 1..6: note = ring structure
GLWGHK

SEQ ID NO: 117 - protein, 6 aa, synthetic construct
  source 1..6: note = ring structure
GLVGHK

SEQ ID NO: 118 - protein, 6 aa, synthetic construct
  source 1..6: note = ring structure
GMAGHK

SEQ ID NO: 119 - protein, 6 aa, synthetic construct
  source 1..6: note = ring structure
GMGGHK

SEQ ID NO: 120 - protein, 6 aa, synthetic construct
  source 1..6: note = ring structure
GMIGHK

SEQ ID NO: 121 - protein, 6 aa, synthetic construct
  source 1..6: note = ring structure
GMLGHK

SEQ ID NO: 122 - protein, 6 aa, synthetic construct
  source 1..6: note = ring structure
GMMGHK

SEQ ID NO: 123 - protein, 6 aa, synthetic construct
  source 1..6: note = ring structure
GMFGHK

SEQ ID NO: 124 - protein, 6 aa, synthetic construct
  source 1..6: note = ring structure
GMPGHK

SEQ ID NO: 125 - protein, 6 aa, synthetic construct
  source 1..6: note = ring structure
GMWGHK

SEQ ID NO: 126 - protein, 6 aa, synthetic construct
  source 1..6: note = ring structure
GMVGHK

SEQ ID NO: 127 - protein, 6 aa, synthetic construct
  source 1..6: note = ring structure
GFAGHK

SEQ ID NO: 128 - protein, 6 aa, synthetic construct
  source 1..6: note = ring structure
GFGGHK

SEQ ID NO: 129 - protein, 6 aa, synthetic construct
  source 1..6: note = ring structure
GFIGHK

SEQ ID NO: 130 - protein, 6 aa, synthetic construct
  source 1..6: note = ring structure
GFLGHK

SEQ ID NO: 131 - protein, 6 aa, synthetic construct
GFMGHK

SEQ ID NO: 132 - protein, 6 aa, synthetic construct
  source 1..6: note = ring structure
GFFGHK

SEQ ID NO: 133 - protein, 6 aa, synthetic construct
  source 1..6: note = ring structure
GFPGHK

SEQ ID NO: 134 - protein, 6 aa, synthetic construct
  source 1..6: note = ring structure
GFWGHK

SEQ ID NO: 135 - protein, 6 aa, synthetic construct
  source 1..6: note = ring structure
GFVGHK

SEQ ID NO: 136 - protein, 6 aa, synthetic construct
  source 1..6: note = ring structure
GPAGHK

SEQ ID NO: 137 - protein, 6 aa, synthetic construct
  source 1..6: note = ring structure
GPGGHK

SEQ ID NO: 138 - protein, 6 aa, synthetic construct
  source 1..6: note = ring structure
GPIGHK

SEQ ID NO: 139 - protein, 6 aa, synthetic construct
  source 1..6: note = ring structure
GPLGHK

SEQ ID NO: 140 - protein, 6 aa, synthetic construct
  source 1..6: note = ring structure
GPMGHK

SEQ ID NO: 141 - protein, 6 aa, synthetic construct
  source 1..6: note = ring structure
GPFGHK

SEQ ID NO: 142 - protein, 6 aa, synthetic construct
  source 1..6: note = ring structure
GPPGHK

SEQ ID NO: 143 - protein, 6 aa, synthetic construct
  source 1..6: note = ring structure
GPWGHK

SEQ ID NO: 144 - protein, 6 aa, synthetic construct
  source 1..6: note = ring structure
GPVGHK

SEQ ID NO: 145 - protein, 6 aa, synthetic construct
  source 1..6: note = ring structure
GWAGHK

SEQ ID NO: 146 - protein, 6 aa, synthetic construct
  source 1..6: note = ring structure
GWGGHK

SEQ ID NO: 147 - protein, 6 aa, synthetic construct
  source 1..6: note = ring structure
GWIGHK

SEQ ID NO: 148 - protein, 6 aa, synthetic construct
  source 1..6: note = ring structure
GWLGHK

SEQ ID NO: 149 - protein, 6 aa, synthetic construct
  source 1..6: note = ring structure
GWMGHK

SEQ ID NO: 150 - protein, 6 aa, synthetic construct
  source 1..6: note = ring structure
GWFGHK

SEQ ID NO: 151 - protein, 6 aa, synthetic construct
  source 1..6: note = ring structure
GWPGHK

SEQ ID NO: 152 - protein, 6 aa, synthetic construct
  source 1..6: note = ring structure
GWWGHK

SEQ ID NO: 153 - protein, 6 aa, synthetic construct
  source 1..6: note = ring structure
GWVGHK

SEQ ID NO: 154 - protein, 6 aa, synthetic construct
  source 1..6: note = ring structure
GVAGHK

SEQ ID NO: 155 - protein, 6 aa, synthetic construct
  source 1..6: note = ring structure
GVGGHK

SEQ ID NO: 156 - protein, 6 aa, synthetic construct
  source 1..6: note = ring structure
GVIGHK

SEQ ID NO: 157 - protein, 6 aa, synthetic construct
  source 1..6: note = ring structure
GVLGHK

SEQ ID NO: 158 - protein, 6 aa, synthetic construct
  source 1..6: note = ring structure
GVMGHK

SEQ ID NO: 159 - protein, 6 aa, synthetic construct
  source 1..6: note = ring structure
GVFGHK

SEQ ID NO: 160 - protein, 6 aa, synthetic construct
  source 1..6: note = ring structure
GVPGHK

SEQ ID NO: 161 - protein, 6 aa, synthetic construct
  source 1..6: note = ring structure
GVWGHK

SEQ ID NO: 162 - protein, 6 aa, synthetic construct
  source 1..6: note = ring structure
GVVGHK

SEQ ID NO: 163 - protein, 6 aa, synthetic construct
  source 1..6: note = ring structure
IAAGHK

SEQ ID NO: 164 - protein, 6 aa, synthetic construct
  source 1..6: note = ring structure
IAGGHK

SEQ ID NO: 165 - protein, 6 aa, synthetic construct
  source 1..6: note = ring structure
IAIGHK

SEQ ID NO: 166 - protein, 6 aa, synthetic construct
  source 1..6: note = ring structure
IALGHK

SEQ ID NO: 167 - protein, 6 aa, synthetic construct
  source 1..6: note = ring structure
IAMGHK

SEQ ID NO: 168 - protein, 6 aa, synthetic construct
  source 1..6: note = ring structure
IAFGHK

SEQ ID NO: 169 - protein, 6 aa, synthetic construct
  source 1..6: note = ring structure
IAPGHK

SEQ ID NO: 170 - protein, 6 aa, synthetic construct
  source 1..6: note = ring structure
IAWGHK

SEQ ID NO: 171 - protein, 6 aa, synthetic construct
  source 1..6: note = ring structure
IAVGHK

SEQ ID NO: 172 - protein, 6 aa, synthetic construct
  source 1..6: note = ring structure
IGAGHK

SEQ ID NO: 173 - protein, 6 aa, synthetic construct
  source 1..6: note = ring structure
IGGGHK

SEQ ID NO: 174 - protein, 6 aa, synthetic construct
  source 1..6: note = ring structure
IGIGHK

SEQ ID NO: 175 - protein, 6 aa, synthetic construct
  source 1..6: note = ring structure
IGLGHK

SEQ ID NO: 176 - protein, 6 aa, synthetic construct
  source 1..6: note = ring structure
IGMGHK

SEQ ID NO: 177 - protein, 6 aa, synthetic construct
  source 1..6: note = ring structure
IGFGHK

SEQ ID NO: 178 - protein, 6 aa, synthetic construct
  source 1..6: note = ring structure
IGPGHK

SEQ ID NO: 179 - protein, 6 aa, synthetic construct
  source 1..6: note = ring structure
IGWGHK

SEQ ID NO: 180 - protein, 6 aa, synthetic construct
  source 1..6: note = ring structure
IGVGHK

SEQ ID NO: 181 - protein, 6 aa, synthetic construct
  source 1..6: note = ring structure
IIAGHK

SEQ ID NO: 182 - protein, 6 aa, synthetic construct
  source 1..6: note = ring structure
IIGGHK

SEQ ID NO: 183 - protein, 6 aa, synthetic construct
  source 1..6: note = ring structure
IIIGHK

SEQ ID NO: 184 - protein, 6 aa, synthetic construct
  source 1..6: note = ring structure
IILGHK

SEQ ID NO: 185 - protein, 6 aa, synthetic construct
  source 1..6: note = ring structure
IIMGHK

SEQ ID NO: 186 - protein, 6 aa, synthetic construct
  source 1..6: note = ring structure
IIFGHK

SEQ ID NO: 187 - protein, 6 aa, synthetic construct
  source 1..6: note = ring structure
IIPGHK

SEQ ID NO: 188 - protein, 6 aa, synthetic construct
  source 1..6: note = ring structure
IIWGHK

SEQ ID NO: 189 - protein, 6 aa, synthetic construct
  source 1..6: note = ring structure
IIVGHK

SEQ ID NO: 190 - protein, 6 aa, synthetic construct
  source 1..6: note = ring structure
ILAGHK

SEQ ID NO: 191 - protein, 6 aa, synthetic construct
  source 1..6: note = ring structure
ILGGHK

SEQ ID NO: 192 - protein, 6 aa, synthetic construct
  source 1..6: note = ring structure
ILIGHK

SEQ ID NO: 193 - protein, 6 aa, synthetic construct
  source 1..6: note = ring structure
ILLGHK

SEQ ID NO: 194 - protein, 6 aa, synthetic construct
  source 1..6: note = ring structure
ILMGHK

SEQ ID NO: 195 - protein, 6 aa, synthetic construct
  source 1..6: note = ring structure
ILFGHK

SEQ ID NO: 196 - protein, 6 aa, synthetic construct
  source 1..6: note = ring structure
ILPGHK

SEQ ID NO: 197 - protein, 6 aa, synthetic construct
  source 1..6: note = ring structure
ILWGHK

SEQ ID NO: 198 - protein, 6 aa, synthetic construct
  source 1..6: note = ring structure
ILVGHK

SEQ ID NO: 199 - protein, 6 aa, synthetic construct
  source 1..6: note = ring structure
IMAGHK

SEQ ID NO: 200 - protein, 6 aa, synthetic construct
  source 1..6: note = ring structure
IMGGHK

SEQ ID NO: 201 - protein, 6 aa, synthetic construct
  source 1..6: note = ring structure
IMIGHK

SEQ ID NO: 202 - protein, 6 aa, synthetic construct
  source 1..6: note = ring structure
IMLGHK

SEQ ID NO: 203 - protein, 6 aa, synthetic construct
  source 1..6: note = ring structure
IMMGHK

SEQ ID NO: 204 - protein, 6 aa, synthetic construct
  source 1..6: note = ring structure
IMFGHK

SEQ ID NO: 205 - protein, 6 aa, synthetic construct
  source 1..6: note = ring structure
IMPGHK

SEQ ID NO: 206 - protein, 6 aa, synthetic construct
  source 1..6: note = ring structure
IMWGHK

SEQ ID NO: 207 - protein, 6 aa, synthetic construct
  source 1..6: note = ring structure
IMVGHK

SEQ ID NO: 208 - protein, 6 aa, synthetic construct
  source 1..6: note = ring structure
IFAGHK

SEQ ID NO: 209 - protein, 6 aa, synthetic construct
  source 1..6: note = ring structure
IFGGHK

SEQ ID NO: 210 - protein, 6 aa, synthetic construct
  source 1..6: note = ring structure
IFIGHK

SEQ ID NO: 211 - protein, 6 aa, synthetic construct
  source 1..6: note = ring structure
IFLGHK

SEQ ID NO: 212 - protein, 6 aa, synthetic construct
  source 1..6: note = ring structure
IFMGHK

SEQ ID NO: 213 - protein, 6 aa, synthetic construct
  source 1..6: note = ring structure
IFFGHK

SEQ ID NO: 214 - protein, 6 aa, synthetic construct
  source 1..6: note = ring structure
IFPGHK

SEQ ID NO: 215 - protein, 6 aa, synthetic construct
  source 1..6: note = ring structure
IFWGHK

SEQ ID NO: 216 - protein, 6 aa, synthetic construct
  source 1..6: note = ring structure
IFVGHK

SEQ ID NO: 217 - protein, 6 aa, synthetic construct
  source 1..6: note = ring structure
IPAGHK

SEQ ID NO: 218 - protein, 6 aa, synthetic construct
  source 1..6: note = ring structure
IPGGHK

SEQ ID NO: 219 - protein, 6 aa, synthetic construct
  source 1..6: note = ring structure
IPIGHK

SEQ ID NO: 220 - protein, 6 aa, synthetic construct
  source 1..6: note = ring structure
IPLGHK

SEQ ID NO: 221 - protein, 6 aa, synthetic construct
  source 1..6: note = ring structure
IPMGHK

SEQ ID NO: 222 - protein, 6 aa, synthetic construct
  source 1..6: note = ring structure
IPFGHK

SEQ ID NO: 223 - protein, 6 aa, synthetic construct
  source 1..6: note = ring structure
IPPGHK

SEQ ID NO: 224 - protein, 6 aa, synthetic construct
  source 1..6: note = ring structure
IPWGHK

SEQ ID NO: 225 - protein, 6 aa, synthetic construct
  source 1..6: note = ring structure
IPVGHK

SEQ ID NO: 226 - protein, 6 aa, synthetic construct
  source 1..6: note = ring structure
IWAGHK

SEQ ID NO: 227 - protein, 6 aa, synthetic construct
  source 1..6: note = ring structure
IWGGHK

SEQ ID NO: 228 - protein, 6 aa, synthetic construct
  source 1..6: note = ring structure
IWIGHK

SEQ ID NO: 229 - protein, 6 aa, synthetic construct
  source 1..6: note = ring structure
IWLGHK

SEQ ID NO: 230 - protein, 6 aa, synthetic construct
  source 1..6: note = ring structure
IWMGHK

SEQ ID NO: 231 - protein, 6 aa, synthetic construct
  source 1..6: note = ring structure
IWFGHK

SEQ ID NO: 232 - protein, 6 aa, synthetic construct
  source 1..6: note = ring structure
IWPGHK

SEQ ID NO: 233 - protein, 6 aa, synthetic construct
  source 1..6: note = ring structure
IWWGHK

SEQ ID NO: 234 - protein, 6 aa, synthetic construct
  source 1..6: note = ring structure
IWVGHK

SEQ ID NO: 235 - protein, 6 aa, synthetic construct
  source 1..6: note = ring structure
IVAGHK

SEQ ID NO: 236 - protein, 6 aa, synthetic construct
  source 1..6: note = ring structure
IVGGHK

SEQ ID NO: 237 - protein, 6 aa, synthetic construct
  source 1..6: note = ring structure
IVIGHK

SEQ ID NO: 238 - protein, 6 aa, synthetic construct
  source 1..6: note = ring structure
IVLGHK

SEQ ID NO: 239 - protein, 6 aa, synthetic construct
  source 1..6: note = ring structure
IVMGHK

SEQ ID NO: 240 - protein, 6 aa, synthetic construct
  source 1..6: note = ring structure
IVFGHK

SEQ ID NO: 241 - protein, 6 aa, synthetic construct
  source 1..6: note = ring structure
IVPGHK

SEQ ID NO: 242 - protein, 6 aa, synthetic construct
  source 1..6: note = ring structure
IVWGHK

SEQ ID NO: 243 - protein, 6 aa, synthetic construct
  source 1..6: note = ring structure
IVVGHK

SEQ ID NO: 244 - protein, 6 aa, synthetic construct
  source 1..6: note = ring structure
LAAGHK

SEQ ID NO: 245 - protein, 6 aa, synthetic construct
  source 1..6: note = ring structure
LAGGHK

SEQ ID NO: 246 - protein, 6 aa, synthetic construct
  source 1..6: note = ring structure
LAIGHK

SEQ ID NO: 247 - protein, 6 aa, synthetic construct
  source 1..6: note = ring structure
LALGHK

SEQ ID NO: 248 - protein, 6 aa, synthetic construct
  source 1..6: note = ring structure
LAMGHK

SEQ ID NO: 249 - protein, 6 aa, synthetic construct
  source 1..6: note = ring structure
LAFGHK

SEQ ID NO: 250 - protein, 6 aa, synthetic construct
  source 1..6: note = ring structure
LAPGHK

SEQ ID NO: 251 - protein, 6 aa, synthetic construct
  source 1..6: note = ring structure
LAWGHK

SEQ ID NO: 252 - protein, 6 aa, synthetic construct
  source 1..6: note = ring structure
LAVGHK

SEQ ID NO: 253 - protein, 6 aa, synthetic construct
  source 1..6: note = ring structure
LGAGHK

SEQ ID NO: 254 - protein, 6 aa, synthetic construct
  source 1..6: note = ring structure
LGGGHK

SEQ ID NO: 255 - protein, 6 aa, synthetic construct
  source 1..6: note = ring structure
LGIGHK

SEQ ID NO: 256 - protein, 6 aa, synthetic construct
  source 1..6: note = ring structure
LGLGHK

SEQ ID NO: 257 - protein, 6 aa, synthetic construct
  source 1..6: note = ring structure
LGMGHK

SEQ ID NO: 258 - protein, 6 aa, synthetic construct
  source 1..6: note = ring structure
LGFGHK

SEQ ID NO: 259 - protein, 6 aa, synthetic construct
  source 1..6: note = ring structure
LGPGHK

SEQ ID NO: 260 - protein, 6 aa, synthetic construct
  source 1..6: note = ring structure
LGWGHK

SEQ ID NO: 261 - protein, 6 aa, synthetic construct
  source 1..6: note = ring structure
LGVGHK

SEQ ID NO: 262 - protein, 6 aa, synthetic construct
  source 1..6: note = ring structure
LIAGHK

SEQ ID NO: 263 - protein, 6 aa, synthetic construct
  source 1..6: note = ring structure
LIGGHK

SEQ ID NO: 264 - protein, 6 aa, synthetic construct
  source 1..6: note = ring structure
LIIGHK

SEQ ID NO: 265 - protein, 6 aa, synthetic construct
  source 1..6: note = ring structure
LILGHK

SEQ ID NO: 266 - protein, 6 aa, synthetic construct
  source 1..6: note = ring structure
LIMGHK

SEQ ID NO: 267 - protein, 6 aa, synthetic construct
  source 1..6: note = ring structure
LIFGHK

SEQ ID NO: 268 - protein, 6 aa, synthetic construct
  source 1..6: note = ring structure
LIPGHK

SEQ ID NO: 269 - protein, 6 aa, synthetic construct
  source 1..6: note = ring structure
LIWGHK

SEQ ID NO: 270 - protein, 6 aa, synthetic construct
  source 1..6: note = ring structure
LIVGHK

SEQ ID NO: 271 - protein, 6 aa, synthetic construct
  source 1..6: note = ring structure
LLAGHK

SEQ ID NO: 272 - protein, 6 aa, synthetic construct
  source 1..6: note = ring structure
LLGGHK

SEQ ID NO: 273 - protein, 6 aa, synthetic construct
  source 1..6: note = ring structure
LLIGHK

SEQ ID NO: 274 - protein, 6 aa, synthetic construct
  source 1..6: note = ring structure
LLLGHK

SEQ ID NO: 275 - protein, 6 aa, synthetic construct
  source 1..6: note = ring structure
LLMGHK

SEQ ID NO: 276 - protein, 6 aa, synthetic construct
  source 1..6: note = ring structure
LLFGHK

SEQ ID NO: 277 - protein, 6 aa, synthetic construct
  source 1..6: note = ring structure
LLPGHK

SEQ ID NO: 278 - protein, 6 aa, synthetic construct
  source 1..6: note = ring structure
LLWGHK

SEQ ID NO: 279 - protein, 6 aa, synthetic construct
  source 1..6: note = ring structure
LLVGHK

SEQ ID NO: 280 - protein, 6 aa, synthetic construct
  source 1..6: note = ring structure
LMAGHK

SEQ ID NO: 281 - protein, 6 aa, synthetic construct
  source 1..6: note = ring structure
LMGGHK

SEQ ID NO: 282 - protein, 6 aa, synthetic construct
  source 1..6: note = ring structure
LMIGHK

SEQ ID NO: 283 - protein, 6 aa, synthetic construct
  source 1..6: note = ring structure
LMLGHK

SEQ ID NO: 284 - protein, 6 aa, synthetic construct
  source 1..6: note = ring structure
LMMGHK

SEQ ID NO: 285 - protein, 6 aa, synthetic construct
  source 1..6: note = ring structure
LMFGHK

SEQ ID NO: 286 - protein, 6 aa, synthetic construct
  source 1..6: note = ring structure
LMPGHK

SEQ ID NO: 287 - protein, 6 aa, synthetic construct
  source 1..6: note = ring structure
LMWGHK

SEQ ID NO: 288 - protein, 6 aa, synthetic construct
  source 1..6: note = ring structure
LMVGHK

SEQ ID NO: 289 - protein, 6 aa, synthetic construct
  source 1..6: note = ring structure
LFAGHK

SEQ ID NO: 290 - protein, 6 aa, synthetic construct
  source 1..6: note = ring structure
LFGGHK

SEQ ID NO: 291 - protein, 6 aa, synthetic construct
  source 1..6: note = ring structure
LFIGHK

SEQ ID NO: 292 - protein, 6 aa, synthetic construct
  source 1..6: note = ring structure
LFLGHK

SEQ ID NO: 293 - protein, 6 aa, synthetic construct
  source 1..6: note = ring structure
LFMGHK

SEQ ID NO: 294 - protein, 6 aa, synthetic construct
  source 1..6: note = ring structure
LFFGHK

SEQ ID NO: 295 - protein, 6 aa, synthetic construct
  source 1..6: note = ring structure
LFPGHK

SEQ ID NO: 296 - protein, 6 aa, synthetic construct
  source 1..6: note = ring structure
LFWGHK

SEQ ID NO: 297 - protein, 6 aa, synthetic construct
  source 1..6: note = ring structure
LFVGHK

SEQ ID NO: 298 - protein, 6 aa, synthetic construct
  source 1..6: note = ring structure
LPAGHK

SEQ ID NO: 299 - protein, 6 aa, synthetic construct
  source 1..6: note = ring structure
LPGGHK

SEQ ID NO: 300 - protein, 6 aa, synthetic construct
  source 1..6: note = ring structure
LPIGHK

SEQ ID NO: 301 - protein, 6 aa, synthetic construct
  source 1..6: note = ring structure
LPLGHK

SEQ ID NO: 302 - protein, 6 aa, synthetic construct
  source 1..6: note = ring structure
LPMGHK

SEQ ID NO: 303 - protein, 6 aa, synthetic construct
  source 1..6: note = ring structure
LPFGHK

SEQ ID NO: 304 - protein, 6 aa, synthetic construct
  source 1..6: note = ring structure
LPPGHK

SEQ ID NO: 305 - protein, 6 aa, synthetic construct
  source 1..6: note = ring structure
LPWGHK

SEQ ID NO: 306 - protein, 6 aa, synthetic construct
  source 1..6: note = ring structure
LPVGHK

SEQ ID NO: 307 - protein, 6 aa, synthetic construct
  source 1..6: note = ring structure
LWAGHK

SEQ ID NO: 308 - protein, 6 aa, synthetic construct
  source 1..6: note = ring structure
LWGGHK

SEQ ID NO: 309 - protein, 6 aa, synthetic construct
  source 1..6: note = ring structure
LWIGHK

SEQ ID NO: 310 - protein, 6 aa, synthetic construct
  source 1..6: note = ring structure
LWLGHK

SEQ ID NO: 311 - protein, 6 aa, synthetic construct
  source 1..6: note = ring structure
LWMGHK

SEQ ID NO: 312 - protein, 6 aa, synthetic construct
  source 1..6: note = ring structure
LWFGHK

SEQ ID NO: 313 - protein, 6 aa, synthetic construct
  source 1..6: note = ring structure
LWPGHK

SEQ ID NO: 314 - protein, 6 aa, synthetic construct
  source 1..6: note = ring structure
LWWGHK

SEQ ID NO: 315 - protein, 6 aa, synthetic construct
  source 1..6: note = ring structure
LWVGHK

SEQ ID NO: 316 - protein, 6 aa, synthetic construct
  source 1..6: note = ring structure
LVAGHK

SEQ ID NO: 317 - protein, 6 aa, synthetic construct
  source 1..6: note = ring structure
LVGGHK

SEQ ID NO: 318 - protein, 6 aa, synthetic construct
  source 1..6: note = ring structure
LVIGHK

SEQ ID NO: 319 - protein, 6 aa, synthetic construct
  source 1..6: note = ring structure
LVLGHK

SEQ ID NO: 320 - protein, 6 aa, synthetic construct
  source 1..6: note = ring structure
LVMGHK

SEQ ID NO: 321 - protein, 6 aa, synthetic construct
  source 1..6: note = ring structure
LVFGHK

SEQ ID NO: 322 - protein, 6 aa, synthetic construct
  source 1..6: note = ring structure
LVPGHK

SEQ ID NO: 323 - protein, 6 aa, synthetic construct
  source 1..6: note = ring structure
LVWGHK

SEQ ID NO: 324 - protein, 6 aa, synthetic construct
  source 1..6: note = ring structure
LVVGHK

SEQ ID NO: 325 - protein, 6 aa, synthetic construct
  source 1..6: note = ring structure
MAAGHK

SEQ ID NO: 326 - protein, 6 aa, synthetic construct
  source 1..6: note = ring structure
MAGGHK

SEQ ID NO: 327 - protein, 6 aa, synthetic construct
  source 1..6: note = ring structure
MAIGHK

SEQ ID NO: 328 - protein, 6 aa, synthetic construct
  source 1..6: note = ring structure
MALGHK

SEQ ID NO: 329 - protein, 6 aa, synthetic construct
  source 1..6: note = ring structure
MAMGHK

SEQ ID NO: 330 - protein, 6 aa, synthetic construct
  source 1..6: note = ring structure
MAFGHK

SEQ ID NO: 331 - protein, 6 aa, synthetic construct
  source 1..6: note = ring structure
MAPGHK

SEQ ID NO: 332 - protein, 6 aa, synthetic construct
  source 1..6: note = ring structure
MAWGHK

SEQ ID NO: 333 - protein, 6 aa, synthetic construct
  source 1..6: note = ring structure
MAVGHK

SEQ ID NO: 334 - protein, 6 aa, synthetic construct
  source 1..6: note = ring structure
MGAGHK

SEQ ID NO: 335 - protein, 6 aa, synthetic construct
  source 1..6: note = ring structure
MGGGHK

SEQ ID NO: 336 - protein, 6 aa, synthetic construct
  source 1..6: note = ring structure
MGIGHK

SEQ ID NO: 337 - protein, 6 aa, synthetic construct
  source 1..6: note = ring structure
MGLGHK

SEQ ID NO: 338 - protein, 6 aa, synthetic construct
  source 1..6: note = ring structure
MGMGHK

SEQ ID NO: 339 - protein, 6 aa, synthetic construct
  source 1..6: note = ring structure
MGFGHK

SEQ ID NO: 340 - protein, 6 aa, synthetic construct
  source 1..6: note = ring structure
MGPGHK

SEQ ID NO: 341 - protein, 6 aa, synthetic construct
  source 1..6: note = ring structure
MGWGHK

SEQ ID NO: 342 - protein, 6 aa, synthetic construct
  source 1..6: note = ring structure
MGVGHK

SEQ ID NO: 343 - protein, 6 aa, synthetic construct
  source 1..6: note = ring structure
MIAGHK

SEQ ID NO: 344 - protein, 6 aa, synthetic construct
  source 1..6: note = ring structure
MIGGHK

SEQ ID NO: 345 - protein, 6 aa, synthetic construct
  source 1..6: note = ring structure
MIIGHK

SEQ ID NO: 346 - protein, 6 aa, synthetic construct
  source 1..6: note = ring structure
MILGHK

SEQ ID NO: 347 - protein, 6 aa, synthetic construct
  source 1..6: note = ring structure
MIMGHK

SEQ ID NO: 348 - protein, 6 aa, synthetic construct
  source 1..6: note = ring structure
MIFGHK

SEQ ID NO: 349 - protein, 6 aa, synthetic construct
  source 1..6: note = ring structure
MIPGHK

SEQ ID NO: 350 - protein, 6 aa, synthetic construct
  source 1..6: note = ring structure
MIWGHK

SEQ ID NO: 351 - protein, 6 aa, synthetic construct
  source 1..6: note = ring structure
MIVGHK

SEQ ID NO: 352 - protein, 6 aa, synthetic construct
  source 1..6: note = ring structure
MLAGHK

SEQ ID NO: 353 - protein, 6 aa, synthetic construct
  source 1..6: note = ring structure
MLGGHK

SEQ ID NO: 354 - protein, 6 aa, synthetic construct
  source 1..6: note = ring structure
MLIGHK

SEQ ID NO: 355 - protein, 6 aa, synthetic construct
  source 1..6: note = ring structure
MLLGHK

SEQ ID NO: 356 - protein, 6 aa, synthetic construct
  source 1..6: note = ring structure
MLMGHK

SEQ ID NO: 357 - protein, 6 aa, synthetic construct
  source 1..6: note = ring structure
MLFGHK

SEQ ID NO: 358 - protein, 6 aa, synthetic construct
  source 1..6: note = ring structure
MLPGHK

SEQ ID NO: 359 - protein, 6 aa, synthetic construct
  source 1..6: note = ring structure
MLWGHK

SEQ ID NO: 360 - protein, 6 aa, synthetic construct
  source 1..6: note = ring structure
MLVGHK

SEQ ID NO: 361 - protein, 6 aa, synthetic construct
  source 1..6: note = ring structure
MMAGHK

SEQ ID NO: 362 - protein, 6 aa, synthetic construct
  source 1..6: note = ring structure
MMGGHK

SEQ ID NO: 363 - protein, 6 aa, synthetic construct
  source 1..6: note = ring structure
MMIGHK

SEQ ID NO: 364 - protein, 6 aa, synthetic construct
  source 1..6: note = ring structure
MMLGHK

SEQ ID NO: 365 - protein, 6 aa, synthetic construct
  source 1..6: note = ring structure
MMMGHK

SEQ ID NO: 366 - protein, 6 aa, synthetic construct
  source 1..6: note = ring structure
MMFGHK

SEQ ID NO: 367 - protein, 6 aa, synthetic construct
  source 1..6: note = ring structure
MMPGHK

SEQ ID NO: 368 - protein, 6 aa, synthetic construct
  source 1..6: note = ring structure
MMWGHK

SEQ ID NO: 369 - protein, 6 aa, synthetic construct
  source 1..6: note = ring structure
MMVGHK

SEQ ID NO: 370 - protein, 6 aa, synthetic construct
  source 1..6: note = ring structure
MFAGHK

SEQ ID NO: 371 - protein, 6 aa, synthetic construct
  source 1..6: note = ring structure
MFGGHK

SEQ ID NO: 372 - protein, 6 aa, synthetic construct
  source 1..6: note = ring structure
MFIGHK

SEQ ID NO: 373 - protein, 6 aa, synthetic construct
  source 1..6: note = ring structure
MFLGHK

SEQ ID NO: 374 - protein, 6 aa, synthetic construct
  source 1..6: note = ring structure
MFMGHK

SEQ ID NO: 375 - protein, 6 aa, synthetic construct
  source 1..6: note = ring structure
MFFGHK

SEQ ID NO: 376 - protein, 6 aa, synthetic construct
  source 1..6: note = ring structure
MFPGHK

SEQ ID NO: 377 - protein, 6 aa, synthetic construct
  source 1..6: note = ring structure
MFWGHK

SEQ ID NO: 378 - protein, 6 aa, synthetic construct
  source 1..6: note = ring structure
MFVGHK

SEQ ID NO: 379 - protein, 6 aa, synthetic construct
  source 1..6: note = ring structure
MPAGHK

SEQ ID NO: 380 - protein, 6 aa, synthetic construct
  source 1..6: note = ring structure
MPGGHK

SEQ ID NO: 381 - protein, 6 aa, synthetic construct
  source 1..6: note = ring structure
MPIGHK

SEQ ID NO: 382 - protein, 6 aa, synthetic construct
  source 1..6: note = ring structure
MPLGHK

SEQ ID NO: 383 - protein, 6 aa, synthetic construct
  source 1..6: note = ring structure
MPMGHK

SEQ ID NO: 384 - protein, 6 aa, synthetic construct
  source 1..6: note = ring structure
MPFGHK

SEQ ID NO: 385 - protein, 6 aa, synthetic construct
  source 1..6: note = ring structure
MPPGHK

SEQ ID NO: 386 - protein, 6 aa, synthetic construct
  source 1..6: note = ring structure
MPWGHK

SEQ ID NO: 387 - protein, 6 aa, synthetic construct
  source 1..6: note = ring structure
MPVGHK

SEQ ID NO: 388 - protein, 6 aa, synthetic construct
  source 1..6: note = ring structure
MWAGHK

SEQ ID NO: 389 - protein, 6 aa, synthetic construct
  source 1..6: note = ring structure
MWGGHK

SEQ ID NO: 390 - protein, 6 aa, synthetic construct
  source 1..6: note = ring structure
MWIGHK

SEQ ID NO: 391 - protein, 6 aa, synthetic construct
  source 1..6: note = ring structure
MWLGHK

SEQ ID NO: 392 - protein, 6 aa, synthetic construct
  source 1..6: note = ring structure
MWMGHK

SEQ ID NO: 393 - protein, 6 aa, synthetic construct
  source 1..6: note = ring structure
MWFGHK

SEQ ID NO: 394 - protein, 6 aa, synthetic construct
  source 1..6: note = ring structure
MWPGHK

SEQ ID NO: 395 - protein, 6 aa, synthetic construct
  source 1..6: note = ring structure
MWWGHK

SEQ ID NO: 396 - protein, 6 aa, synthetic construct
  source 1..6: note = ring structure
MWVGHK

SEQ ID NO: 397 - protein, 6 aa, synthetic construct
  source 1..6: note = ring structure
MVAGHK

SEQ ID NO: 398 - protein, 6 aa, synthetic construct
  source 1..6: note = ring structure
MVGGHK

SEQ ID NO: 399 - protein, 6 aa, synthetic construct
  source 1..6: note = ring structure
MVIGHK

SEQ ID NO: 400 - protein, 6 aa, synthetic construct
  source 1..6: note = ring structure
MVLGHK

SEQ ID NO: 401 - protein, 6 aa, synthetic construct
  source 1..6: note = ring structure
MVMGHK

SEQ ID NO: 402 - protein, 6 aa, synthetic construct
  source 1..6: note = ring structure
MVFGHK

SEQ ID NO: 403 - protein, 6 aa, synthetic construct
  source 1..6: note = ring structure
MVPGHK

SEQ ID NO: 404 - protein, 6 aa, synthetic construct
  source 1..6: note = ring structure
MVWGHK

SEQ ID NO: 405 - protein, 6 aa, synthetic construct
  source 1..6: note = ring structure
MVVGHK

SEQ ID NO: 406 - protein, 6 aa, synthetic construct
  source 1..6: note = ring structure
FAAGHK

SEQ ID NO: 407 - protein, 6 aa, synthetic construct
  source 1..6: note = ring structure
FAGGHK

SEQ ID NO: 408 - protein, 6 aa, synthetic construct
  source 1..6: note = ring structure
FAIGHK

SEQ ID NO: 409 - protein, 6 aa, synthetic construct
  source 1..6: note = ring structure
FALGHK

SEQ ID NO: 410 - protein, 6 aa, synthetic construct
  source 1..6: note = ring structure
FAMGHK

SEQ ID NO: 411 - protein, 6 aa, synthetic construct
  source 1..6: note = ring structure
FAFGHK

SEQ ID NO: 412 - protein, 6 aa, synthetic construct
  source 1..6: note = ring structure
FAPGHK

SEQ ID NO: 413 - protein, 6 aa, synthetic construct
  source 1..6: note = ring structure
FAWGHK

SEQ ID NO: 414 - protein, 6 aa, synthetic construct
  source 1..6: note = ring structure
FAVGHK

SEQ ID NO: 415 - protein, 6 aa, synthetic construct
  source 1..6: note = ring structure
FGAGHK

SEQ ID NO: 416 - protein, 6 aa, synthetic construct
  source 1..6: note = ring structure
FGGGHK

SEQ ID NO: 417 - protein, 6 aa, synthetic construct
  source 1..6: note = ring structure
FGIGHK

SEQ ID NO: 418 - protein, 6 aa, synthetic construct
  source 1..6: note = ring structure
FGLGHK

SEQ ID NO: 419 - protein, 6 aa, synthetic construct
  source 1..6: note = ring structure
FGMGHK

SEQ ID NO: 420 - protein, 6 aa, synthetic construct
  source 1..6: note = ring structure
FGFGHK

SEQ ID NO: 421 - protein, 6 aa, synthetic construct
  source 1..6: note = ring structure
FGPGHK

SEQ ID NO: 422 - protein, 6 aa, synthetic construct
  source 1..6: note = ring structure
FGWGHK

SEQ ID NO: 423 - protein, 6 aa, synthetic construct
  source 1..6: note = ring structure
FGVGHK

SEQ ID NO: 424 - protein, 6 aa, synthetic construct
  source 1..6: note = ring structure
FIAGHK

SEQ ID NO: 425 - protein, 6 aa, synthetic construct
  source 1..6: note = ring structure
FIGGHK

SEQ ID NO: 426 - protein, 6 aa, synthetic construct
  source 1..6: note = ring structure
FIIGHK

SEQ ID NO: 427 - protein, 6 aa, synthetic construct
  source 1..6: note = ring structure
FILGHK

SEQ ID NO: 428 - protein, 6 aa, synthetic construct
  source 1..6: note = ring structure
FIMGHK

SEQ ID NO: 429 - protein, 6 aa, synthetic construct
  source 1..6: note = ring structure
FIFGHK

SEQ ID NO: 430 - protein, 6 aa, synthetic construct
  source 1..6: note = ring structure
FIPGHK

SEQ ID NO: 431 - protein, 6 aa, synthetic construct
  source 1..6: note = ring structure
FIWGHK

SEQ ID NO: 432 - protein, 6 aa, synthetic construct
  source 1..6: note = ring structure
FIVGHK

SEQ ID NO: 433 - protein, 6 aa, synthetic construct
  source 1..6: note = ring structure
FLAGHK

SEQ ID NO: 434 - protein, 6 aa, synthetic construct
  source 1..6: note = ring structure
FLGGHK

SEQ ID NO: 435 - protein, 6 aa, synthetic construct
  source 1..6: note = ring structure
FLIGHK

SEQ ID NO: 436 - protein, 6 aa, synthetic construct
  source 1..6: note = ring structure
FLLGHK

SEQ ID NO: 437 - protein, 6 aa, synthetic construct
  source 1..6: note = ring structure
FLMGHK

SEQ ID NO: 438 - protein, 6 aa, synthetic construct
  source 1..6: note = ring structure
FLFGHK

SEQ ID NO: 439 - protein, 6 aa, synthetic construct
  source 1..6: note = ring structure
FLPGHK

SEQ ID NO: 440 - protein, 6 aa, synthetic construct
  source 1..6: note = ring structure
FLWGHK

SEQ ID NO: 441 - protein, 6 aa, synthetic construct
  source 1..6: note = ring structure
FLVGHK

SEQ ID NO: 442 - protein, 6 aa, synthetic construct
  source 1..6: note = ring structure
FMAGHK

SEQ ID NO: 443 - protein, 6 aa, synthetic construct
  source 1..6: note = ring structure
FMGGHK

SEQ ID NO: 444 - protein, 6 aa, synthetic construct
  source 1..6: note = ring structure
FMIGHK

SEQ ID NO: 445 - protein, 6 aa, synthetic construct
  source 1..6: note = ring structure
FMLGHK

SEQ ID NO: 446 - protein, 6 aa, synthetic construct
  source 1..6: note = ring structure
FMMGHK

SEQ ID NO: 447 - protein, 6 aa, synthetic construct
  source 1..6: note = ring structure
FMFGHK

SEQ ID NO: 448 - protein, 6 aa, synthetic construct
  source 1..6: note = ring structure
FMPGHK

SEQ ID NO: 449 - protein, 6 aa, synthetic construct
  source 1..6: note = ring structure
FMWGHK

SEQ ID NO: 450 - protein, 6 aa, synthetic construct
  source 1..6: note = ring structure
FMVGHK

SEQ ID NO: 451 - protein, 6 aa, synthetic construct
  source 1..6: note = ring structure
FFAGHK

SEQ ID NO: 452 - protein, 6 aa, synthetic construct
  source 1..6: note = ring structure
FFGGHK

SEQ ID NO: 453 - protein, 6 aa, synthetic construct
  source 1..6: note = ring structure
FFIGHK

SEQ ID NO: 454 - protein, 6 aa, synthetic construct
  source 1..6: note = ring structure
FFLGHK

SEQ ID NO: 455 - protein, 6 aa, synthetic construct
  source 1..6: note = ring structure
FFMGHK

SEQ ID NO: 456 - protein, 6 aa, synthetic construct
  source 1..6: note = ring structure
FFFGHK

SEQ ID NO: 457 - protein, 6 aa, synthetic construct
  source 1..6: note = ring structure
FFPGHK

SEQ ID NO: 458 - protein, 6 aa, synthetic construct
  source 1..6: note = ring structure
FFWGHK

SEQ ID NO: 459 - protein, 6 aa, synthetic construct
  source 1..6: note = ring structure
FFVGHK

SEQ ID NO: 460 - protein, 6 aa, synthetic construct
  source 1..6: note = ring structure
FPAGHK

SEQ ID NO: 461 - protein, 6 aa, synthetic construct
  source 1..6: note = ring structure
FPGGHK

SEQ ID NO: 462 - protein, 6 aa, synthetic construct
  source 1..6: note = ring structure
FPIGHK

SEQ ID NO: 463 - protein, 6 aa, synthetic construct
  source 1..6: note = ring structure
FPLGHK

SEQ ID NO: 464 - protein, 6 aa, synthetic construct
  source 1..6: note = ring structure
FPMGHK

SEQ ID NO: 465 - protein, 6 aa, synthetic construct
  source 1..6: note = ring structure
FPFGHK

SEQ ID NO: 466 - protein, 6 aa, synthetic construct
  source 1..6: note = ring structure
FPPGHK

SEQ ID NO: 467 - protein, 6 aa, synthetic construct
  source 1..6: note = ring structure
FPWGHK

SEQ ID NO: 468 - protein, 6 aa, synthetic construct
  source 1..6: note = ring structure
FPVGHK

SEQ ID NO: 469 - protein, 6 aa, synthetic construct
  source 1..6: note = ring structure
FWAGHK

SEQ ID NO: 470 - protein, 6 aa, synthetic construct
  source 1..6: note = ring structure
FWGGHK

SEQ ID NO: 471 - protein, 6 aa, synthetic construct
  source 1..6: note = ring structure
FWIGHK

SEQ ID NO: 472 - protein, 6 aa, synthetic construct
  source 1..6: note = ring structure
FWLGHK

SEQ ID NO: 473 - protein, 6 aa, synthetic construct
  source 1..6: note = ring structure
FWMGHK

SEQ ID NO: 474 - protein, 6 aa, synthetic construct
  source 1..6: note = ring structure
FWFGHK

SEQ ID NO: 475 - protein, 6 aa, synthetic construct
  source 1..6: note = ring structure
FWPGHK

SEQ ID NO: 476 - protein, 6 aa, synthetic construct
  source 1..6: note = ring structure
FWWGHK

SEQ ID NO: 477 - protein, 6 aa, synthetic construct
  source 1..6: note = ring structure
FWVGHK

SEQ ID NO: 478 - protein, 6 aa, synthetic construct
  source 1..6: note = ring structure
FVAGHK

SEQ ID NO: 479 - protein, 6 aa, synthetic construct
  source 1..6: note = ring structure
FVGGHK

SEQ ID NO: 480 - protein, 6 aa, synthetic construct
  source 1..6: note = ring structure
FVIGHK

SEQ ID NO: 481 - protein, 6 aa, synthetic construct
  source 1..6: note = ring structure
FVLGHK

SEQ ID NO: 482 - protein, 6 aa, synthetic construct
  source 1..6: note = ring structure
FVMGHK

SEQ ID NO: 483 - protein, 6 aa, synthetic construct
  source 1..6: note = ring structure
FVFGHK

SEQ ID NO: 484 - protein, 6 aa, synthetic construct
  source 1..6: note = ring structure
FVPGHK

SEQ ID NO: 485 - protein, 6 aa, synthetic construct
  source 1..6: note = ring structure
FVWGHK

SEQ ID NO: 486 - protein, 6 aa, synthetic construct
  source 1..6: note = ring structure
FVVGHK

SEQ ID NO: 487 - protein, 6 aa, synthetic construct
  source 1..6: note = ring structure
PAAGHK

SEQ ID NO: 488 - protein, 6 aa, synthetic construct
  source 1..6: note = ring structure
PAGGHK

SEQ ID NO: 489 - protein, 6 aa, synthetic construct
  source 1..6: note = ring structure
PAIGHK

SEQ ID NO: 490 - protein, 6 aa, synthetic construct
  source 1..6: note = ring structure
PALGHK

SEQ ID NO: 491 - protein, 6 aa, synthetic construct
  source 1..6: note = ring structure
PAMGHK

SEQ ID NO: 492 - protein, 6 aa, synthetic construct
  source 1..6: note = ring structure
PAFGHK

SEQ ID NO: 493 - protein, 6 aa, synthetic construct
  source 1..6: note = ring structure
PAPGHK

SEQ ID NO: 494 - protein, 6 aa, synthetic construct
  source 1..6: note = ring structure
PAWGHK

SEQ ID NO: 495 - protein, 6 aa, synthetic construct
  source 1..6: note = ring structure
PAVGHK

SEQ ID NO: 496 - protein, 6 aa, synthetic construct
  source 1..6: note = ring structure
PGAGHK

SEQ ID NO: 497 - protein, 6 aa, synthetic construct
  source 1..6: note = ring structure
PGGGHK

SEQ ID NO: 498 - protein, 6 aa, synthetic construct
  source 1..6: note = ring structure
PGIGHK

SEQ ID NO: 499 - protein, 6 aa, synthetic construct
  source 1..6: note = ring structure
PGLGHK

SEQ ID NO: 500 - protein, 6 aa, synthetic construct
  source 1..6: note = ring structure
PGMGHK

SEQ ID NO: 501 - protein, 6 aa, synthetic construct
  source 1..6: note = ring structure
PGFGHK

SEQ ID NO: 502 - protein, 6 aa, synthetic construct
  source 1..6: note = ring structure
PGPGHK

SEQ ID NO: 503 - protein, 6 aa, synthetic construct
  source 1..6: note = ring structure
PGWGHK

SEQ ID NO: 504 - protein, 6 aa, synthetic construct
  source 1..6: note = ring structure
PGVGHK

SEQ ID NO: 505 - protein, 6 aa, synthetic construct
  source 1..6: note = ring structure
PIAGHK

SEQ ID NO: 506 - protein, 6 aa, synthetic construct
  source 1..6: note = ring structure
PIGGHK

SEQ ID NO: 507 - protein, 6 aa, synthetic construct
  source 1..6: note = ring structure
PIIGHK

SEQ ID NO: 508 - protein, 6 aa, synthetic construct
  source 1..6: note = ring structure
PILGHK

SEQ ID NO: 509 - protein, 6 aa, synthetic construct
  source 1..6: note = ring structure
PIMGHK

SEQ ID NO: 510 - protein, 6 aa, synthetic construct
  source 1..6: note = ring structure
PIFGHK

SEQ ID NO: 511 - protein, 6 aa, synthetic construct
  source 1..6: note = ring structure
PIPGHK

SEQ ID NO: 512 - protein, 6 aa, synthetic construct
  source 1..6: note = ring structure
PIWGHK

SEQ ID NO: 513 - protein, 6 aa, synthetic construct
  source 1..6: note = ring structure
PIVGHK

SEQ ID NO: 514 - protein, 6 aa, synthetic construct
  source 1..6: note = ring structure
PLAGHK

SEQ ID NO: 515 - protein, 6 aa, synthetic construct
  source 1..6: note = ring structure
PLGGHK

SEQ ID NO: 516 - protein, 6 aa, synthetic construct
  source 1..6: note = ring structure
PLIGHK

SEQ ID NO: 517 - protein, 6 aa, synthetic construct
  source 1..6: note = ring structure
PLLGHK

SEQ ID NO: 518 - protein, 6 aa, synthetic construct
  source 1..6: note = ring structure
PLMGHK

SEQ ID NO: 519 - protein, 6 aa, synthetic construct
  source 1..6: note = ring structure
PLFGHK

SEQ ID NO: 520 - protein, 6 aa, synthetic construct
  source 1..6: note = ring structure
PLPGHK

SEQ ID NO: 521 - protein, 6 aa, synthetic construct
  source 1..6: note = ring structure
PLWGHK

SEQ ID NO: 522 - protein, 6 aa, synthetic construct
  source 1..6: note = ring structure
PLVGHK

SEQ ID NO: 523 - protein, 6 aa, synthetic construct
  source 1..6: note = ring structure
PMAGHK

SEQ ID NO: 524 - protein, 6 aa, synthetic construct
  source 1..6: note = ring structure
PMGGHK

SEQ ID NO: 525 - protein, 6 aa, synthetic construct
  source 1..6: note = ring structure
PMIGHK

SEQ ID NO: 526 - protein, 6 aa, synthetic construct
  source 1..6: note = ring structure
PMLGHK

SEQ ID NO: 527 - protein, 6 aa, synthetic construct
  source 1..6: note = ring structure
PMMGHK

SEQ ID NO: 528 - protein, 6 aa, synthetic construct
  source 1..6: note = ring structure
PMFGHK

SEQ ID NO: 529 - protein, 6 aa, synthetic construct
  source 1..6: note = ring structure
PMPGHK

SEQ ID NO: 530 - protein, 6 aa, synthetic construct
  source 1..6: note = ring structure
PMWGHK

SEQ ID NO: 531 - protein, 6 aa, synthetic construct
  source 1..6: note = ring structure
PMVGHK

SEQ ID NO: 532 - protein, 6 aa, synthetic construct
  source 1..6: note = ring structure
PFAGHK

SEQ ID NO: 533 - protein, 6 aa, synthetic construct
  source 1..6: note = ring structure
PFGGHK

SEQ ID NO: 534 - protein, 6 aa, synthetic construct
  source 1..6: note = ring structure
PFIGHK

SEQ ID NO: 535 - protein, 6 aa, synthetic construct
  source 1..6: note = ring structure
PFLGHK

SEQ ID NO: 536 - protein, 6 aa, synthetic construct
  source 1..6: note = ring structure
PFMGHK

SEQ ID NO: 537 - protein, 6 aa, synthetic construct
  source 1..6: note = ring structure
PFFGHK

SEQ ID NO: 538 - protein, 6 aa, synthetic construct
  source 1..6: note = ring structure
PFPGHK

SEQ ID NO: 539 - protein, 6 aa, synthetic construct
  source 1..6: note = ring structure
PFWGHK

SEQ ID NO: 540 - protein, 6 aa, synthetic construct
  source 1..6: note = ring structure
PFVGHK

SEQ ID NO: 541 - protein, 6 aa, synthetic construct
  source 1..6: note = ring structure
PPAGHK

SEQ ID NO: 542 - protein, 6 aa, synthetic construct
  source 1..6: note = ring structure
PPGGHK

SEQ ID NO: 543 - protein, 6 aa, synthetic construct
  source 1..6: note = ring structure
PPIGHK

SEQ ID NO: 544 - protein, 6 aa, synthetic construct
  source 1..6: note = ring structure
PPLGHK

SEQ ID NO: 545 - protein, 6 aa, synthetic construct
  source 1..6: note = ring structure
PPMGHK

SEQ ID NO: 546 - protein, 6 aa, synthetic construct
  source 1..6: note = ring structure
PPFGHK

SEQ ID NO: 547 - protein, 6 aa, synthetic construct
  source 1..6: note = ring structure
PPPGHK

SEQ ID NO: 548 - protein, 6 aa, synthetic construct
  source 1..6: note = ring structure
PPWGHK

SEQ ID NO: 549 - protein, 6 aa, synthetic construct
  source 1..6: note = ring structure
PPVGHK

SEQ ID NO: 550 - protein, 6 aa, synthetic construct
  source 1..6: note = ring structure
PWAGHK

SEQ ID NO: 551 - protein, 6 aa, synthetic construct
  source 1..6: note = ring structure
PWGGHK

SEQ ID NO: 552 - protein, 6 aa, synthetic construct
  source 1..6: note = ring structure
PWIGHK

SEQ ID NO: 553 - protein, 6 aa, synthetic construct
  source 1..6: note = ring structure
PWLGHK

SEQ ID NO: 554 - protein, 6 aa, synthetic construct
  source 1..6: note = ring structure
PWMGHK

SEQ ID NO: 555 - protein, 6 aa, synthetic construct
  source 1..6: note = ring structure
PWFGHK

SEQ ID NO: 556 - protein, 6 aa, synthetic construct
  source 1..6: note = ring structure
PWPGHK

SEQ ID NO: 557 - protein, 6 aa, synthetic construct
  source 1..6: note = ring structure
PWWGHK

SEQ ID NO: 558 - protein, 6 aa, synthetic construct
  source 1..6: note = ring structure
PWVGHK

SEQ ID NO: 559 - protein, 6 aa, synthetic construct
  source 1..6: note = ring structure
PVAGHK

SEQ ID NO: 560 - protein, 6 aa, synthetic construct
  source 1..6: note = ring structure
PVGGHK

SEQ ID NO: 561 - protein, 6 aa, synthetic construct
  source 1..6: note = ring structure
PVIGHK

SEQ ID NO: 562 - protein, 6 aa, synthetic construct
  source 1..6: note = ring structure
PVLGHK

SEQ ID NO: 563 - protein, 6 aa, synthetic construct
  source 1..6: note = ring structure
PVMGHK

SEQ ID NO: 564 - protein, 6 aa, synthetic construct
  source 1..6: note = ring structure
PVFGHK

SEQ ID NO: 565 - protein, 6 aa, synthetic construct
  source 1..6: note = ring structure
PVPGHK

SEQ ID NO: 566 - protein, 6 aa, synthetic construct
  source 1..6: note = ring structure
PVWGHK

SEQ ID NO: 567 - protein, 6 aa, synthetic construct
  source 1..6: note = ring structure
PVVGHK

SEQ ID NO: 568 - protein, 6 aa, synthetic construct
  source 1..6: note = ring structure
WAAGHK

SEQ ID NO: 569 - protein, 6 aa, synthetic construct
  source 1..6: note = ring structure
WAGGHK

SEQ ID NO: 570 - protein, 6 aa, synthetic construct
  source 1..6: note = ring structure
WAIGHK

SEQ ID NO: 571 - protein, 6 aa, synthetic construct
  source 1..6: note = ring structure
WALGHK

SEQ ID NO: 572 - protein, 6 aa, synthetic construct
  source 1..6: note = ring structure
WAMGHK

SEQ ID NO: 573 - protein, 6 aa, synthetic construct
  source 1..6: note = ring structure
WAFGHK

SEQ ID NO: 574 - protein, 6 aa, synthetic construct
  source 1..6: note = ring structure
WAPGHK

SEQ ID NO: 575 - protein, 6 aa, synthetic construct
  source 1..6: note = ring structure
WAWGHK

SEQ ID NO: 576 - protein, 6 aa, synthetic construct
  source 1..6: note = ring structure
WAVGHK

SEQ ID NO: 577 - protein, 6 aa, synthetic construct
  source 1..6: note = ring structure
WGAGHK

SEQ ID NO: 578 - protein, 6 aa, synthetic construct
  source 1..6: note = ring structure
WGGGHK

SEQ ID NO: 579 - protein, 6 aa, synthetic construct
  source 1..6: note = ring structure
WGIGHK

SEQ ID NO: 580 - protein, 6 aa, synthetic construct
  source 1..6: note = ring structure
WGLGHK

SEQ ID NO: 581 - protein, 6 aa, synthetic construct
  source 1..6: note = ring structure
WGMGHK

SEQ ID NO: 582 - protein, 6 aa, synthetic construct
  source 1..6: note = ring structure
WGFGHK

SEQ ID NO: 583 - protein, 6 aa, synthetic construct
  source 1..6: note = ring structure
WGPGHK

SEQ ID NO: 584 - protein, 6 aa, synthetic construct
  source 1..6: note = ring structure
WGWGHK

SEQ ID NO: 585 - protein, 6 aa, synthetic construct
  source 1..6: note = ring structure
WGVGHK

SEQ ID NO: 586 - protein, 6 aa, synthetic construct
  source 1..6: note = ring structure
WIAGHK

SEQ ID NO: 587 - protein, 6 aa, synthetic construct
  source 1..6: note = ring structure
WIGGHK

SEQ ID NO: 588 - protein, 6 aa, synthetic construct
  source 1..6: note = ring structure
WIIGHK

SEQ ID NO: 589 - protein, 6 aa, synthetic construct
  source 1..6: note = ring structure
WILGHK

SEQ ID NO: 590 - protein, 6 aa, synthetic construct
  source 1..6: note = ring structure
WIMGHK

SEQ ID NO: 591 - protein, 6 aa, synthetic construct
  source 1..6: note = ring structure
WIFGHK

SEQ ID NO: 592 - protein, 6 aa, synthetic construct
  source 1..6: note = ring structure
WIPGHK

SEQ ID NO: 593 - protein, 6 aa, synthetic construct
  source 1..6: note = ring structure
WIWGHK

SEQ ID NO: 594 - protein, 6 aa, synthetic construct
  source 1..6: note = ring structure
WIVGHK

SEQ ID NO: 595 - protein, 6 aa, synthetic construct
  source 1..6: note = ring structure
WLAGHK

SEQ ID NO: 596 - protein, 6 aa, synthetic construct
  source 1..6: note = ring structure
WLGGHK

SEQ ID NO: 597 - protein, 6 aa, synthetic construct
  source 1..6: note = ring structure
WLIGHK

SEQ ID NO: 598 - protein, 6 aa, synthetic construct
  source 1..6: note = ring structure
WLLGHK

SEQ ID NO: 599 - protein, 6 aa, synthetic construct
  source 1..6: note = ring structure
WLMGHK

SEQ ID NO: 600 - protein, 6 aa, synthetic construct
  source 1..6: note = ring structure
WLFGHK

SEQ ID NO: 601 - protein, 6 aa, synthetic construct
  source 1..6: note = ring structure
WLPGHK

SEQ ID NO: 602 - protein, 6 aa, synthetic construct
  source 1..6: note = ring structure
WLWGHK

SEQ ID NO: 603 - protein, 6 aa, synthetic construct
  source 1..6: note = ring structure
WLVGHK

SEQ ID NO: 604 - protein, 6 aa, synthetic construct
  source 1..6: note = ring structure
WMAGHK

SEQ ID NO: 605 - protein, 6 aa, synthetic construct
  source 1..6: note = ring structure
WMGGHK

SEQ ID NO: 606 - protein, 6 aa, synthetic construct
  source 1..6: note = ring structure
WMIGHK

SEQ ID NO: 607 - protein, 6 aa, synthetic construct
  source 1..6: note = ring structure
WMLGHK

SEQ ID NO: 608 - protein, 6 aa, synthetic construct
  source 1..6: note = ring structure
WMMGHK

SEQ ID NO: 609 - protein, 6 aa, synthetic construct
  source 1..6: note = ring structure
WMFGHK

SEQ ID NO: 610 - protein, 6 aa, synthetic construct
  source 1..6: note = ring structure
WMPGHK

SEQ ID NO: 611 - protein, 6 aa, synthetic construct
  source 1..6: note = ring structure
WMWGHK

SEQ ID NO: 612 - protein, 6 aa, synthetic construct
  source 1..6: note = ring structure
WMVGHK

SEQ ID NO: 613 - protein, 6 aa, synthetic construct
  source 1..6: note = ring structure
WFAGHK

SEQ ID NO: 614 - protein, 6 aa, synthetic construct
  source 1..6: note = ring structure
WFGGHK

SEQ ID NO: 615 - protein, 6 aa, synthetic construct
  source 1..6: note = ring structure
WFIGHK

SEQ ID NO: 616 - protein, 6 aa, synthetic construct
  source 1..6: note = ring structure
WFLGHK

SEQ ID NO: 617 - protein, 6 aa, synthetic construct
  source 1..6: note = ring structure
WFMGHK

SEQ ID NO: 618 - protein, 6 aa, synthetic construct
  source 1..6: note = ring structure
WFFGHK

SEQ ID NO: 619 - protein, 6 aa, synthetic construct
  source 1..6: note = ring structure
WFPGHK

SEQ ID NO: 620 - protein, 6 aa, synthetic construct
  source 1..6: note = ring structure
WFWGHK

SEQ ID NO: 621 - protein, 6 aa, synthetic construct
  source 1..6: note = ring structure
WFVGHK

SEQ ID NO: 622 - protein, 6 aa, synthetic construct
  source 1..6: note = ring structure
WPAGHK

SEQ ID NO: 623 - protein, 6 aa, synthetic construct
  source 1..6: note = ring structure
WPGGHK

SEQ ID NO: 624 - protein, 6 aa, synthetic construct
  source 1..6: note = ring structure
WPIGHK

SEQ ID NO: 625 - protein, 6 aa, synthetic construct
  source 1..6: note = ring structure
WPLGHK

SEQ ID NO: 626 - protein, 6 aa, synthetic construct
  source 1..6: note = ring structure
WPMGHK

SEQ ID NO: 627 - protein, 6 aa, synthetic construct
  source 1..6: note = ring structure
WPFGHK

SEQ ID NO: 628 - protein, 6 aa, synthetic construct
  source 1..6: note = ring structure
WPPGHK

SEQ ID NO: 629 - protein, 6 aa, synthetic construct
  source 1..6: note = ring structure
WPWGHK

SEQ ID NO: 630 - protein, 6 aa, synthetic construct
  source 1..6: note = ring structure
WPVGHK

SEQ ID NO: 631 - protein, 6 aa, synthetic construct
  source 1..6: note = ring structure
WWAGHK

SEQ ID NO: 632 - protein, 6 aa, synthetic construct
  source 1..6: note = ring structure
WWGGHK

SEQ ID NO: 633 - protein, 6 aa, synthetic construct
  source 1..6: note = ring structure; note = ring structure
WWIGHK

SEQ ID NO: 634 - protein, 6 aa, synthetic construct
  source 1..6: note = ring structure; note = ring structure
WWLGHK

SEQ ID NO: 635 - protein, 6 aa, synthetic construct
  source 1..6: note = ring structure
WWMGHK

SEQ ID NO: 636 - protein, 6 aa, synthetic construct
  source 1..6: note = ring structure
WWFGHK

SEQ ID NO: 637 - protein, 6 aa, synthetic construct
  source 1..6: note = ring structure
WWPGHK

SEQ ID NO: 638 - protein, 6 aa, synthetic construct
  source 1..6: note = ring structure
WWWGHK

SEQ ID NO: 639 - protein, 6 aa, synthetic construct
  source 1..6: note = ring structure
WWVGHK

SEQ ID NO: 640 - protein, 6 aa, synthetic construct
  source 1..6: note = ring structure
WVAGHK

SEQ ID NO: 641 - protein, 6 aa, synthetic construct
  source 1..6: note = ring structure
WVGGHK

SEQ ID NO: 642 - protein, 6 aa, synthetic construct
  source 1..6: note = ring structure
WVIGHK

SEQ ID NO: 643 - protein, 6 aa, synthetic construct
  source 1..6: note = ring structure
WVLGHK

SEQ ID NO: 644 - protein, 6 aa, synthetic construct
  source 1..6: note = ring structure
WVMGHK

SEQ ID NO: 645 - protein, 6 aa, synthetic construct
  source 1..6: note = ring structure
WVFGHK

SEQ ID NO: 646 - protein, 6 aa, synthetic construct
  source 1..6: note = ring structure
WVPGHK

SEQ ID NO: 647 - protein, 6 aa, synthetic construct
  source 1..6: note = ring structure
WVWGHK

SEQ ID NO: 648 - protein, 6 aa, synthetic construct
  source 1..6: note = ring structure
WVVGHK

SEQ ID NO: 649 - protein, 6 aa, synthetic construct
  source 1..6: note = ring structure
VAAGHK

SEQ ID NO: 650 - protein, 6 aa, synthetic construct
  source 1..6: note = ring structure
VAGGHK

SEQ ID NO: 651 - protein, 6 aa, synthetic construct
  source 1..6: note = ring structure
VAIGHK

SEQ ID NO: 652 - protein, 6 aa, synthetic construct
  source 1..6: note = ring structure
VALGHK

SEQ ID NO: 653 - protein, 6 aa, synthetic construct
  source 1..6: note = ring structure
VAMGHK

SEQ ID NO: 654 - protein, 6 aa, synthetic construct
  source 1..6: note = ring structure
VAFGHK

SEQ ID NO: 655 - protein, 6 aa, synthetic construct
  source 1..6: note = ring structure
VAPGHK

SEQ ID NO: 656 - protein, 6 aa, synthetic construct
  source 1..6: note = ring structure
VAWGHK

SEQ ID NO: 657 - protein, 6 aa, synthetic construct
  source 1..6: note = ring structure
VAVGHK

SEQ ID NO: 658 - protein, 6 aa, synthetic construct
  source 1..6: note = ring structure
VGAGHK

SEQ ID NO: 659 - protein, 6 aa, synthetic construct
  source 1..6: note = ring structure
VGGGHK

SEQ ID NO: 660 - protein, 6 aa, synthetic construct
  source 1..6: note = ring structure
VGIGHK

SEQ ID NO: 661 - protein, 6 aa, synthetic construct
  source 1..6: note = ring structure
VGLGHK

SEQ ID NO: 662 - protein, 6 aa, synthetic construct
  source 1..6: note = ring structure
VGMGHK

SEQ ID NO: 663 - protein, 6 aa, synthetic construct
  source 1..6: note = ring structure
VGFGHK

SEQ ID NO: 664 - protein, 6 aa, synthetic construct
  source 1..6: note = ring structure
VGPGHK

SEQ ID NO: 665 - protein, 6 aa, synthetic construct
  source 1..6: note = ring structure
VGWGHK

SEQ ID NO: 666 - protein, 6 aa, synthetic construct
  source 1..6: note = ring structure
VGVGHK

SEQ ID NO: 667 - protein, 6 aa, synthetic construct
  source 1..6: note = ring structure
VIAGHK

SEQ ID NO: 668 - protein, 6 aa, synthetic construct
  source 1..6: note = ring structure
VIGGHK

SEQ ID NO: 669 - protein, 6 aa, synthetic construct
  source 1..6: note = ring structure
VIIGHK

SEQ ID NO: 670 - protein, 6 aa, synthetic construct
  source 1..6: note = ring structure
VILGHK

SEQ ID NO: 671 - protein, 6 aa, synthetic construct
  source 1..6: note = ring structure
VIMGHK

SEQ ID NO: 672 - protein, 6 aa, synthetic construct
  source 1..6: note = ring structure
VIFGHK

SEQ ID NO: 673 - protein, 6 aa, synthetic construct
  source 1..6: note = ring structure
VIPGHK

SEQ ID NO: 674 - protein, 6 aa, synthetic construct
  source 1..6: note = ring structure
VIWGHK

SEQ ID NO: 675 - protein, 6 aa, synthetic construct
  source 1..6: note = ring structure
VIVGHK

SEQ ID NO: 676 - protein, 6 aa, synthetic construct
  source 1..6: note = ring structure
VLAGHK

SEQ ID NO: 677 - protein, 6 aa, synthetic construct
  source 1..6: note = ring structure
VLGGHK

SEQ ID NO: 678 - protein, 6 aa, synthetic construct
  source 1..6: note = ring structure
VLIGHK

SEQ ID NO: 679 - protein, 6 aa, synthetic construct
  source 1..6: note = ring structure
VLLGHK

SEQ ID NO: 680 - protein, 6 aa, synthetic construct
  source 1..6: note = ring structure
VLMGHK

SEQ ID NO: 681 - protein, 6 aa, synthetic construct
  source 1..6: note = ring structure
VLFGHK

SEQ ID NO: 682 - protein, 6 aa, synthetic construct
  source 1..6: note = ring structure
VLPGHK

SEQ ID NO: 683 - protein, 6 aa, synthetic construct
  source 1..6: note = ring structure
VLWGHK

SEQ ID NO: 684 - protein, 6 aa, synthetic construct
  source 1..6: note = ring structure
VLVGHK

SEQ ID NO: 685 - protein, 6 aa, synthetic construct
  source 1..6: note = ring structure
VMAGHK

SEQ ID NO: 686 - protein, 6 aa, synthetic construct
  source 1..6: note = ring structure
VMGGHK

SEQ ID NO: 687 - protein, 6 aa, synthetic construct
  source 1..6: note = ring structure
VMIGHK

SEQ ID NO: 688 - protein, 6 aa, synthetic construct
  source 1..6: note = ring structure
VMLGHK

SEQ ID NO: 689 - protein, 6 aa, synthetic construct
  source 1..6: note = ring structure
VMMGHK

SEQ ID NO: 690 - protein, 6 aa, synthetic construct
  source 1..6: note = ring structure
VMFGHK

SEQ ID NO: 691 - protein, 6 aa, synthetic construct
  source 1..6: note = ring structure
VMPGHK

SEQ ID NO: 692 - protein, 6 aa, synthetic construct
  source 1..6: note = ring structure
VMWGHK

SEQ ID NO: 693 - protein, 6 aa, synthetic construct
  source 1..6: note = ring structure
VMVGHK

SEQ ID NO: 694 - protein, 6 aa, synthetic construct
  source 1..6: note = ring structure
VFAGHK

SEQ ID NO: 695 - protein, 6 aa, synthetic construct
  source 1..6: note = ring structure
VFGGHK

SEQ ID NO: 696 - protein, 6 aa, synthetic construct
  source 1..6: note = ring structure
VFIGHK

SEQ ID NO: 697 - protein, 6 aa, synthetic construct
  source 1..6: note = ring structure
VFLGHK

SEQ ID NO: 698 - protein, 6 aa, synthetic construct
  source 1..6: note = ring structure
VFMGHK

SEQ ID NO: 699 - protein, 6 aa, synthetic construct
  source 1..6: note = ring structure
VFFGHK

SEQ ID NO: 700 - protein, 6 aa, synthetic construct
  source 1..6: note = ring structure
VFPGHK

SEQ ID NO: 701 - protein, 6 aa, synthetic construct
  source 1..6: note = ring structure
VFWGHK

SEQ ID NO: 702 - protein, 6 aa, synthetic construct
  source 1..6: note = ring structure
VFVGHK

SEQ ID NO: 703 - protein, 6 aa, synthetic construct
  source 1..6: note = ring structure
VPAGHK

SEQ ID NO: 704 - protein, 6 aa, synthetic construct
  source 1..6: note = ring structure
VPGGHK

SEQ ID NO: 705 - protein, 6 aa, synthetic construct
  source 1..6: note = ring structure
VPIGHK

SEQ ID NO: 706 - protein, 6 aa, synthetic construct
  source 1..6: note = ring structure
VPLGHK

SEQ ID NO: 707 - protein, 6 aa, synthetic construct
  source 1..6: note = ring structure
VPMGHK

SEQ ID NO: 708 - protein, 6 aa, synthetic construct
  source 1..6: note = ring structure
VPFGHK

SEQ ID NO: 709 - protein, 6 aa, synthetic construct
  source 1..6: note = ring structure
VPPGHK

SEQ ID NO: 710 - protein, 6 aa, synthetic construct
  source 1..6: note = ring structure
VPWGHK

SEQ ID NO: 711 - protein, 6 aa, synthetic construct
  source 1..6: note = ring structure
VPVGHK

SEQ ID NO: 712 - protein, 6 aa, synthetic construct
  source 1..6: note = ring structure
VWAGHK

SEQ ID NO: 713 - protein, 6 aa, synthetic construct
  source 1..6: note = ring structure
VWGGHK

SEQ ID NO: 714 - protein, 6 aa, synthetic construct
  source 1..6: note = ring structure
VWIGHK

SEQ ID NO: 715 - protein, 6 aa, synthetic construct
  source 1..6: note = ring structure
VWLGHK

SEQ ID NO: 716 - protein, 6 aa, synthetic construct
  source 1..6: note = ring structure
VWMGHK

SEQ ID NO: 717 - protein, 6 aa, synthetic construct
  source 1..6: note = ring structure
VWFGHK

SEQ ID NO: 718 - protein, 6 aa, synthetic construct
  source 1..6: note = ring structure
VWPGHK

SEQ ID NO: 719 - protein, 6 aa, synthetic construct
  source 1..6: note = ring structure
VWWGHK

SEQ ID NO: 720 - protein, 6 aa, synthetic construct
  source 1..6: note = ring structure
VWVGHK

SEQ ID NO: 721 - protein, 6 aa, synthetic construct
  source 1..6: note = ring structure
VVAGHK

SEQ ID NO: 722 - protein, 6 aa, synthetic construct
  source 1..6: note = ring structure
VVGGHK

SEQ ID NO: 723 - protein, 6 aa, synthetic construct
  source 1..6: note = ring structure
VVIGHK

SEQ ID NO: 724 - protein, 6 aa, synthetic construct
  source 1..6: note = ring structure
VVLGHK

SEQ ID NO: 725 - protein, 6 aa, synthetic construct
  source 1..6: note = ring structure
VVMGHK

SEQ ID NO: 726 - protein, 6 aa, synthetic construct
  source 1..6: note = ring structure
VVFGHK

SEQ ID NO: 727 - protein, 6 aa, synthetic construct
  source 1..6: note = ring structure
VVPGHK

SEQ ID NO: 728 - protein, 6 aa, synthetic construct
  source 1..6: note = ring structure
VVWGHK

SEQ ID NO: 729 - protein, 6 aa, synthetic construct
  source 1..6: note = ring structure
VVVGHK